European Patent Specification EP 3 851 536 B1, published August 26, 2026. Title: SH3 domain derivatives. Applicant: Next Biomed Therapies Oy. The sequence listing filed with the application follows.

SEQUENCE LISTING (21 sequences)

SEQ ID NO: 1 - protein, 57 aa, Homo sapiens
  NPHP1-SH3
EEYIAVGDFTAQQVGDLTFKKGEILLVIEKKPDGWWIAKDAKGNEGLVPRTYLEPYS

SEQ ID NO: 2 - protein, 57 aa, Homo sapiens
  Tec-SH3
EIVVAMYDFQAAEGHDLRLERGQEYLILEKNDVHWWRARDKYGNEGYIPSNYVTGKK

SEQ ID NO: 3 - protein, 58 aa, Homo sapiens
  Fyn-SH3
TLFVALYDYEARTEDDLSFHKGEKFQILNSSEGDWWEARSLTTGETGYIPSNYVAPVD

SEQ ID NO: 4 - protein, 57 aa, Homo sapiens
  Hck-SH3
IIVVALYDYEAIHHEDLSFQKGDQMVVLEESGEWWKARSLATRKEGYIPSNYVARVD

SEQ ID NO: 5 - protein, 71 aa, Homo sapiens
  Amph-SH3
YKVETLHDFEAANSDELTLQRGDVVLVVPSDSEADQDAGWLVGVKESDWLQYRDLATYKGLFPENFTRRLD

SEQ ID NO: 6 - protein, 64 aa, Homo sapiens
  RIMBP3-SH3
KIMIAALDYDPGDGQMGGQGKGRLALRAGDVVMVYGPMDDQGFYYGELGGHRGLVPAHLLDHMS

SEQ ID NO: 7 - protein, 60 aa, Homo sapiens
  IRTKS-SH3
QKVKTIFPHTAGSNKTLLSFAQGDVITLLIPEEKDGWLYGEHDVSKARGWFPSSYTKLLE

SEQ ID NO: 8 - protein, 58 aa, Homo sapiens
  SNX30-SH3
LKGRALYDFHSENKEEISIQQDEDLVIFSETSLDGWLQGQNSRGETGLFPASYVEIVR

SEQ ID NO: 9 - protein, 56 aa, Homo sapiens
  Eps8L1-SH3
KWVLCNYDFQARNSSELSVKQRDVLEVLDDSRKWWKVRDPAGQEGYVPYNILTPYP

SEQ ID NO: 10 - protein, 59 aa, Homo sapiens
  FISH#5-SH3
DVYVSIADYEGDEETAGFQEGVSMEVLERNPNGWWYCQILDGVKPFKGWVPSNYLEKKN

SEQ ID NO: 11 - protein, 57 aa, Homo sapiens
  CMS#1-SH3
VDYIVEYDYDAVHDDELTIRVGEIIRNVKKLQEEGWLEGELNGRRGMFPDNFVKEIK

SEQ ID NO: 12 - protein, 56 aa, Homo sapiens
  OSTF1-SH3
KVFRALYTFEPRTPDELYFEEGDIIYITDMSDTNWWKGTSKGRTGLIPSNYVAEQA

SEQ ID NO: 13 - protein, 6 aa, Homo sapiens
  RT-loop sequence of NPHP1-SH3
TAQQVG

SEQ ID NO: 14 - DNA, 54 bp, Artificial Sequence
  An oligonucleotide used for the generation of drHck-SH3 library
  variation 20,21,23,24,26,27,29,30,32,33,35,36: /replace="a" /replace="g" /replace="c" /replace="t"
agaacgtgctttccaccagnngnngnngnngnngnnagattcttccagaacgac

SEQ ID NO: 15 - DNA, 58 bp, Artificial Sequence
  An oligonucleotides used for the generation of drHck-SH3 library
  variation 21,22,24,25,27,28,30,31,33,34,36,37: /replace="a" /replace="g" /replace="c" /replace="t"
gtgctttccaccattcaccgnngnngnngnngnngnncagaacgaccatctgatcacc

SEQ ID NO: 16 - protein, 60 aa, Artificial Sequence
  NPHP1-drSH3 sequence with randomized loop residues
EEYIAVGDFCTYTGPDLTFKKGEILLVIERPFAHTDGWWIAKDAKGNEGLVPRTYLEPYS

SEQ ID NO: 17 - protein, 60 aa, Artificial Sequence
  NPHP1-drSH3 sequence with randomized loop residues
EEYIAVGDFQPSMPCDLTFKKGEILLVIEQLQMCLDGWWIAKDAKGNEGLVPRTYLEPYS

SEQ ID NO: 18 - protein, 60 aa, Artificial Sequence
  TEC-drSH3 sequence with randomized loop residues
EIVVAMYDFMSNSVHDLRLERGQEYLILEKQDKRGVHWWRARDKYGNEGYIPSNYVTGKK

SEQ ID NO: 19 - protein, 63 aa, Artificial Sequence
  NPHP1-drSH3 sequence selected from the library of randomized loop residues
EEYIAVGDFYGCDPVDLTFKKGEILLVIEKKPSFVWIPDGWWIAKDAKGNEGLVPRTYLEPYS

SEQ ID NO: 20 - protein, 63 aa, Artificial Sequence
  TEC-drSH3 sequence selected from the library of randomized loop residues
EIVVAMYDFNTSSWWDLRLERGQEYLILEKNSSFKFHDVHWWRARDKYGNEGYIPSNYVTGKK

SEQ ID NO: 21 - protein, 63 aa, Artificial Sequence
  Tec-drSH3 sequence selected from the library of randomized loop residues
EIVVAMYDFHSTPWWDLRLERGQEYLILEKNSSFTLWDVHWWRARDKYGNEGYIPSNYVTGKK